European Patent Specification EP 3 492 585 B1, published February 18, 2026. Title: Method for Preparing Mesenchymal Stem Cells Inhibiting Cancer Proliferation. Applicant: RA, Jeong Chan. The sequence listing filed with the application follows.

SEQUENCE LISTING (26 sequences)

SEQ ID NO: 1 - DNA, 22 bp, Artificial Sequence
  hTRAIL-F
atggctatgatggaggtccagg

SEQ ID NO: 2 - DNA, 23 bp, Artificial Sequence
  hTRAIL-R
tcagctcgttggtaaagtacacg

SEQ ID NO: 3 - DNA, 20 bp, Artificial Sequence
  h Fas L-F
ctggggatgtttcagctctt

SEQ ID NO: 4 - DNA, 21 bp, Artificial Sequence
  h Fas L-R
gtggcctatttgcttctccaa

SEQ ID NO: 5 - DNA, 19 bp, Artificial Sequence
  h CXCR4-F
gcggaaaaccaagacgctc

SEQ ID NO: 6 - DNA, 20 bp, Artificial Sequence
  h CXCR4-R
ttcatgtgcgcgtaactgtc

SEQ ID NO: 7 - DNA, 20 bp, Artificial Sequence
  h VEGF-A-F
tgagcttcctacagcacaac

SEQ ID NO: 8 - DNA, 21 bp, Artificial Sequence
  h VEGF-A-R
gaacgctccaggacttatacc

SEQ ID NO: 9 - DNA, 20 bp, Artificial Sequence
  h Nrf2-F
accagtggatctgccaacta

SEQ ID NO: 10 - DNA, 20 bp, Artificial Sequence
  h Nrf2-R
acgtagccgaagaaacctca

SEQ ID NO: 11 - DNA, 20 bp, Artificial Sequence
  h c-Myc-F
aaggcccccaaggtagttat

SEQ ID NO: 12 - DNA, 20 bp, Artificial Sequence
  h c-Myc-R
ttccgcaacaagtcctcttc

SEQ ID NO: 13 - DNA, 20 bp, Artificial Sequence
  h p21-F
tgtcttgtacccttgtgcct

SEQ ID NO: 14 - DNA, 21 bp, Artificial Sequence
  h p21-R
gcgtttggagtggtagaaatc

SEQ ID NO: 15 - DNA, 19 bp, Artificial Sequence
  h Sox2-F
gcggaaaaccaagacgctc

SEQ ID NO: 16 - DNA, 20 bp, Artificial Sequence
  h Sox2-R
ttcatgtgcgcgtaactgtc

SEQ ID NO: 17 - DNA, 21 bp, Artificial Sequence
  h Nanog-F
tccaacatccrcaacctcagc

SEQ ID NO: 18 - DNA, 20 bp, Artificial Sequence
  h Nanog-R
ccttctgcgtcacaccattg

SEQ ID NO: 19 - DNA, 20 bp, Artificial Sequence
  h Oct4-F
cactgtactcggtccctttc

SEQ ID NO: 20 - DNA, 21 bp, Artificial Sequence
  h Oct4-R
caggcacctcagtttgaatgc

SEQ ID NO: 21 - DNA, 25 bp, Artificial Sequence
  h Bcl2-F
gggtacgataaccgggagatagtga

SEQ ID NO: 22 - DNA, 20 bp, Artificial Sequence
  h Bcl2-R
ggaggagaagatgcccggtg

SEQ ID NO: 23 - DNA, 20 bp, Artificial Sequence
  h PPAR-r-F
ttagatgacagcgacttggc

SEQ ID NO: 24 - DNA, 20 bp, Artificial Sequence
  h PPAR-r-R
ggcttgtagcaggttgtctt

SEQ ID NO: 25 - DNA, 22 bp, Artificial Sequence
  h Apaf 1-F
cttcttccagtgtaaggacagt

SEQ ID NO: 26 - DNA, 20 bp, Artificial Sequence
  h Apaf 1-R
cagcctgccattccatgtat